European Patent Application EP 4 112 632 A1, published January 4, 2023. Title: SYMMETRIC PROTEINS. Applicant: Katholieke Universiteit Leuven. The sequence listing filed with the application follows.

SEQUENCE LISTING (33 sequences)

SEQ ID NO: 1 - DNA, 944 bp, Artificial Sequence
  SAKE protein
  CDS (12)..(935)
gggaattccatatggatggacgtatatacgcggttggcgggtatgatggaagtcccgacggtcatacgcacctgaattctgtcgaagcctacgatcccgagaccgacacttggagtctggttgcccccatgaaaactcgccgttctggtgtaggagttgcggtcctggacggcagaatctatgccgttggcgggtatgatggatcccctgacggccacactcaccttaattcagtggaggcctatgatcccgaaaccgatacctggagcttggtggcccccatgaagacacggcggtcgggcgtcggcgtagcggtcttggatgggagaatatatgcagttggtgggtacgatgggtcgcctgatggacacactcatttgaactccgtagaagcttacgatccggagacggatacatggtctcttgtggcacctatgaaaacccggagatctggcgtcggagtcgccgtattggatggcagaatatacgctgtcgggggctacgacggcagccctgacggtcacactcaccttaattctgtagaggcatacgaccccgaaacagacacgtggagcctggttgctccaatgaaaacacgcagatccggcgtgggggtagcggtgctggatggccgtatctacgcggttggagggtatgacggcagccccgatggtcacacccacctgaatagtgtggaagcgtatgatcctgagacggacacctggtctttggtggctcctatgaaaacgagacgttcaggagtaggagttgcagttttggacggtcgtatttatgcagttgggggatatgacggatccccggacggccacacgcacttgaattcagttgaagcttatgacccagagactgatacctggtcgctggttgctccgatgaaaacgcggcggaacggtgttggcgtggctgtcctttaactcgagcgg

SEQ ID NO: 2 - protein, 307 aa, Artificial Sequence
  Synthetic Construct
MDGRIYAVGGYDGSPDGHTHLNSVEAYDPETDTWSLVAPMKTRRSGVGVAVLDGRIYAVGGYDGSPDGHTHLNSVEAYDPETDTWSLVAPMKTRRSGVGVAVLDGRIYAVGGYDGSPDGHTHLNSVEAYDPETDTWSLVAPMKTRRSGVGVAVLDGRIYAVGGYDGSPDGHTHLNSVEAYDPETDTWSLVAPMKTRRSGVGVAVLDGRIYAVGGYDGSPDGHTHLNSVEAYDPETDTWSLVAPMKTRRSGVGVAVLDGRIYAVGGYDGSPDGHTHLNSVEAYDPETDTWSLVAPMKTRRNGVGVAVL

SEQ ID NO: 3 - DNA, 944 bp, Artificial Sequence
  SAKE protein
  CDS (12)..(935)
gggaattccatatgaatagattgttgtacgctgttggggggtatgatggtagtccagatggccatacccacctgaactccgttgagtgctacgatccagagaccaacgaatggtcgcttgtagcacctatgaatacccgccgttcaggcgttggggtagctgttttaaatcgcctgctgtacgcggttggcgggtacgacggatcccctgatgggcacacccacttgaactctgtagaatgctatgaccctgaaacgaatgagtggtcccttgtcgctcccatgaatacgagacgttcaggagttggagttgcagttttaaaccgccttctttatgcggttggcggttacgacggtagcccagatggacacactcacttgaattctgtggagtgctacgaccctgagacgaacgaatggagtttagttgcaccgatgaatacgcgccggagcggtgtaggtgtagccgtgcttaatcggttactttacgcagtagggggttacgacggatctcctgacggtcacacccacttaaactctgtcgaatgttacgatcctgagactaacgagtggtctttagtcgctcccatgaatacccgccgcagcggcgtaggcgtagcggtacttaaccggttgttgtatgcagttggcgggtacgacgggtcaccggacggccacacgcacctgaactctgtcgaatgttacgaccccgaaacaaatgagtggagcctggtggcccctatgaacactcgcagatcaggagtcggggtagcggtgttaaacagacttctgtatgctgtgggaggctacgatggatccccggacgggcatacccatctgaattcagtggagtgttatgatcccgagacgaacgaatggtcgcttgtagcgcccatgaatacgcggagaagcggtgtcggcgttgcggtcctttaactcgagcgg

SEQ ID NO: 4 - protein, 307 aa, Artificial Sequence
  Synthetic Construct
MNRLLYAVGGYDGSPDGHTHLNSVECYDPETNEWSLVAPMNTRRSGVGVAVLNRLLYAVGGYDGSPDGHTHLNSVECYDPETNEWSLVAPMNTRRSGVGVAVLNRLLYAVGGYDGSPDGHTHLNSVECYDPETNEWSLVAPMNTRRSGVGVAVLNRLLYAVGGYDGSPDGHTHLNSVECYDPETNEWSLVAPMNTRRSGVGVAVLNRLLYAVGGYDGSPDGHTHLNSVECYDPETNEWSLVAPMNTRRSGVGVAVLNRLLYAVGGYDGSPDGHTHLNSVECYDPETNEWSLVAPMNTRRSGVGVAVL

SEQ ID NO: 5 - DNA, 944 bp, Artificial Sequence
  SAKE protein
  CDS (12)..(935)
gggaattccatatgaatggccgcatttatgccgtaggggggtatgacggatccccagacggacatacacatttaaattcggtagaggcatacgacccggaaacggacgagtggtcgtttgtagctcccatgacaacgccacggtccggagtcggggttgccgtgcttaatggccgtatatatgccgtcgggggttacgacggatcgccagatgggcacactcatttgaatagtgttgaagcttacgatccggagacggatgagtggtcatttgttgctccgatgacaaccccgcgtagtggtgttggagttgcagtcctgaacggccggatctatgccgtcggcggttatgacggttctcctgatggacacacgcacttgaattcagtagaggcttacgaccctgaaacagatgaatggtcctttgttgccccgatgactacaccaagatcgggagttggggtggctgtcctgaatgggagaatttatgcggtaggcggatacgatggtagtccagatggccacacacacttaaactccgtcgaggcatacgacccggagacggatgaatggtcattcgttgcaccaatgactacacctcggtccggggtcggcgtggcagtattaaacgggcgtatctatgccgttggtggctacgacggaagtcccgacggccatacgcatctgaactcggtggaagcctatgaccccgaaactgatgaatggagttttgtggcgcccatgacgacgcctcgctccggcgtcggggtagctgtgctgaacgggcggatttacgcggttggtggttatgatggatcccctgacggacatactcacttgaattctgtggaagcttatgacccagagaccgacgagtggtctttcgtggcgccgatgacgacaccccgctcaggagtcggagtggcggtattgtaactcgagcgg

SEQ ID NO: 6 - protein, 307 aa, Artificial Sequence
  Synthetic Construct
MNGRIYAVGGYDGSPDGHTHLNSVEAYDPETDEWSFVAPMTTPRSGVGVAVLNGRIYAVGGYDGSPDGHTHLNSVEAYDPETDEWSFVAPMTTPRSGVGVAVLNGRIYAVGGYDGSPDGHTHLNSVEAYDPETDEWSFVAPMTTPRSGVGVAVLNGRIYAVGGYDGSPDGHTHLNSVEAYDPETDEWSFVAPMTTPRSGVGVAVLNGRIYAVGGYDGSPDGHTHLNSVEAYDPETDEWSFVAPMTTPRSGVGVAVLNGRIYAVGGYDGSPDGHTHLNSVEAYDPETDEWSFVAPMTTPRSGVGVAVL

SEQ ID NO: 7 - DNA, 872 bp, Artificial Sequence
  SAKE protein
  CDS (12)..(863)
gggaattccatatgaatggactgatatacgcggttggcggatatgatggaaacacgcatttaaactctgttgaagcgtatgatcccgaacgcaatgagtggtccttagttgcaccactttcgactcggcggtcgggggtaggggttgcagtattaaatgggcttatttatgcagttggaggctatgatggaaatacacatctgaattctgtggaggcctatgatcccgagcggaatgagtggtctctggtggccccgctgagcactcgccgttcaggggtcggcgtggccgttctgaacgggcttatatatgccgtggggggttacgacggcaacacacacttaaattctgtagaagcttacgatcccgagagaaacgagtggtcccttgtcgctcctttatccacccgcagaagcggtgtgggtgtggctgtattaaacggtctgatttatgccgtagggggatacgacggtaatacacacctgaatagcgttgaggcctatgatccggagcgcaacgaatggtcgttggttgcgcctttgtcaactcgccggtctggtgtgggggtagccgtgttgaacggcctgatatatgcggtgggtgggtatgatggaaacactcacctgaactcggtagaggcgtacgatccagagcgcaacgagtggtctctggtcgccccactgtcgactcgccggtcaggcgttggggttgccgtacttaacggcctgatttatgcggtcggtggttatgacgggaacactcacctgaattccgtggaagcttatgacccagaacgcaatgaatggagtctggttgcacccctgtctactcgtagatcgggggtcggggtagctgtcttgtaactcgagcgg

SEQ ID NO: 8 - protein, 283 aa, Artificial Sequence
  Synthetic Construct
MNGLIYAVGGYDGNTHLNSVEAYDPERNEWSLVAPLSTRRSGVGVAVLNGLIYAVGGYDGNTHLNSVEAYDPERNEWSLVAPLSTRRSGVGVAVLNGLIYAVGGYDGNTHLNSVEAYDPERNEWSLVAPLSTRRSGVGVAVLNGLIYAVGGYDGNTHLNSVEAYDPERNEWSLVAPLSTRRSGVGVAVLNGLIYAVGGYDGNTHLNSVEAYDPERNEWSLVAPLSTRRSGVGVAVLNGLIYAVGGYDGNTHLNSVEAYDPERNEWSLVAPLSTRRSGVGVAVL

SEQ ID NO: 9 - DNA, 876 bp, Artificial Sequence
  SAKE protein
  CDS (10)..(861)
ccaattcatatgttaatttacgctgtgggcggatacgacggcaatacacatttgaacagtgtcgaggcttatgatcctgaacgtaatgagtggtccttggtggcaccgttgtcaacgcgccgttccggggtaggggtagcagtgttaaatggcttgatttatgcggtgggtggttatgacgggaacacccacttaaatagcgttgaggcctatgatccgcatcacaacgaatggagtctggtcgcccctctgagtacccgtcgcagcggagtaggtgttgctgtcttaaatggcttaatttacgcggtcggcggttatgatggaaatacgcacctgaattccgtagaagcttacgatccggaacgcaatgaatggtcattagtggcgccattatccacgcgtcgcagcggagtaggcgtggcggtattaaacggtcttatttacgcagtaggggggtacgacggaaatactcacttaaactccgtagaggcgtatgacccacatcacaatgagtggagcctggttgcgccattgtctacacgccgtagtggcgtcggagttgctgtattaaacgggttaatctatgccgttggtgggtacgatggaaacacacatctgaattcagtggaggcctatgatccagaacgcaacgaatggtctctggtcgcaccgttatctactcgccgtagcggagtgggagtagcagttttgaatggcttgatctacgctgtgggcggttacgacgggaatacccatcttaactctgtcgaggcttacgaccctcatcacaacgaatggtcactggtggcacccttatcgactcgtcgctctggtgtgggggtagcagttcttaatggctaactcgagtacacgagg

SEQ ID NO: 10 - protein, 283 aa, Artificial Sequence
  Synthetic Construct
MLIYAVGGYDGNTHLNSVEAYDPERNEWSLVAPLSTRRSGVGVAVLNGLIYAVGGYDGNTHLNSVEAYDPHHNEWSLVAPLSTRRSGVGVAVLNGLIYAVGGYDGNTHLNSVEAYDPERNEWSLVAPLSTRRSGVGVAVLNGLIYAVGGYDGNTHLNSVEAYDPHHNEWSLVAPLSTRRSGVGVAVLNGLIYAVGGYDGNTHLNSVEAYDPERNEWSLVAPLSTRRSGVGVAVLNGLIYAVGGYDGNTHLNSVEAYDPHHNEWSLVAPLSTRRSGVGVAVLNG

SEQ ID NO: 11 - DNA, 924 bp, Artificial Sequence
  SAKE protein
  CDS (10)..(915)
gatatccatatgaacgggctgatttatgccgttggaggctacgatgggacagggtacaatacccacctgaatagcgtagaggcttatgatccagaacgtaatgagtggtcactggtcgcgcctctttccacgcgccgctcaggcgttggcgtggcggttttgaacggattgatctacgcggttggtggttacgacggtactggctacaatactcacttgaattcggtggaagcttatgaccctgaacgcaatgaatggagtttagtagccccgctgagcacgcgtcgcagtggcgtcggcgttgcggttcttaacggtttgatctatgcggtcggaggatacgacgggacaggttacaacactcatttaaactcagtcgaggcttacgatccagagcgcaacgagtggtccttggttgctcccctttcaactcgtcgctcaggcgtcggggttgcggttttgaacggccttatttacgctgtcggaggttacgacggaacgggttataatacacatcttaatagcgtagaggcgtatgacccggagcgcaatgagtggtctcttgtagcccctcttagcactcgccgctcaggggtgggtgtggctgtactgaatggcctgatttatgcagttggcggatacgacggcacggggtacaacacacacttaaacagtgtggaagcctacgaccctgaacgcaacgagtggtctctggtcgctccgttatcgacgcgccgctcgggagtaggcgtagcagtgctgaatggtttaatctacgctgtgggaggatacgatggcactggatacaatacgcatctgaattccgtcgaagcctacgaccccgagcgtaatgagtggtccttagtcgccccactttcgactcgtcgttctggagtgggggtcgcagtattataactcgagcgg

SEQ ID NO: 12 - protein, 301 aa, Artificial Sequence
  Synthetic Construct
MNGLIYAVGGYDGTGYNTHLNSVEAYDPERNEWSLVAPLSTRRSGVGVAVLNGLIYAVGGYDGTGYNTHLNSVEAYDPERNEWSLVAPLSTRRSGVGVAVLNGLIYAVGGYDGTGYNTHLNSVEAYDPERNEWSLVAPLSTRRSGVGVAVLNGLIYAVGGYDGTGYNTHLNSVEAYDPERNEWSLVAPLSTRRSGVGVAVLNGLIYAVGGYDGTGYNTHLNSVEAYDPERNEWSLVAPLSTRRSGVGVAVLNGLIYAVGGYDGTGYNTHLNSVEAYDPERNEWSLVAPLSTRRSGVGVAVL

SEQ ID NO: 13 - DNA, 978 bp, Artificial Sequence
  SAKE protein
  CDS (10)..(969)
gatatccatatgaatggattgatttacgccgtaggtggttatgatggtagtccagattactcgacaggaacccacttgaattcggtagaagcctacgatccagaacgtaatgaatggtcgttagtggcgccgctgtccacacgtcgttccggggtgggagtagcagtcttgaacggacttatttacgccgtcggggggtatgatggatccccggattacagtactggaacccacctgaatagtgtggaagcctatgatcccgagcgcaatgaatggagtctggttgcacccttaagtacccgtcgttccggcgtcggagtagcagtattgaatggcttgatctacgcggtaggagggtacgacggttctccagactatagtactgggactcaccttaatagcgtcgaggcctacgatcccgaacgtaacgagtggtccttagttgcccccctgtccacacgccgctctggtgtaggcgtagctgtcttgaacgggcttatctacgctgtggggggctatgacggatcgcccgattattccaccggtacgcatttgaatagcgtggaagcttatgacccagagcgtaacgaatggagtttggttgctcctctgagcacccgtcgctctggggtaggtgtcgccgtattgaatggtttgatttatgcagttggcggctacgacggctctccagattacagcactggcacacacctgaattctgtagaggcttatgatccggagcgcaacgaatggtccctggtggctccacttagcacacgccgcagtggggttggagttgcagtgttaaatggactgatctatgccgtagggggttacgatggtagcccggactattctacaggcacccaccttaacagcgtggaagcgtacgacccagaacgcaatgagtggtctctggtagctccgctttccacacgtcgctcaggagtaggagttgctgtattgtaactcgagcgg

SEQ ID NO: 14 - protein, 319 aa, Artificial Sequence
  Synthetic Construct
MNGLIYAVGGYDGSPDYSTGTHLNSVEAYDPERNEWSLVAPLSTRRSGVGVAVLNGLIYAVGGYDGSPDYSTGTHLNSVEAYDPERNEWSLVAPLSTRRSGVGVAVLNGLIYAVGGYDGSPDYSTGTHLNSVEAYDPERNEWSLVAPLSTRRSGVGVAVLNGLIYAVGGYDGSPDYSTGTHLNSVEAYDPERNEWSLVAPLSTRRSGVGVAVLNGLIYAVGGYDGSPDYSTGTHLNSVEAYDPERNEWSLVAPLSTRRSGVGVAVLNGLIYAVGGYDGSPDYSTGTHLNSVEAYDPERNEWSLVAPLSTRRSGVGVAVL

SEQ ID NO: 15 - DNA, 987 bp, Artificial Sequence
  SAKE
  CDS (10)..(978)
gatatccatatgaacgggcttatctatgctgttggcggttatgatggctccccggatgggtctacccatctgaattcggtcgaagcctatgaccccgagcgcaacgaatggtccttagtcgccccgctgagtacacgtcgtagcggagtaggtgttgcggtgcttaacggattgatctatgcggttggtgggtttgcaactctggaaaccgaatccggagagttggtcccgacagaacttaacagtgtagaagcgtatgaccctgaacgtaatgagtggtcgttagtagctcctttatcaacgcgccgtagtggggttggagttgcagttttaaatggactgatctacgcagtaggaggatatgatgggtcgcctgacgggagtacgcaccttaattcggtagaggcgtacgatccagagcgtaacgagtggagtcttgtagcgccactttcaacacgtcgttcgggtgtcggagtggccgttctgaatgggttaatttatgctgtcggagggtttgccacacttgagaccgagagtggagagcttgtgccaacggagttaaactcagtggaagcttatgatcctgagcgcaatgagtggtcactggtcgctcccctgagtactcgccgcagcggagtgggagtagcagtgttaaatggactgatttatgccgtgggcggctatgacgggagtcctgatggtagcacgcatctgaattcggtggaggcctacgatcccgagcgtaacgagtggtccctggtagcgcctctttcgactcgtcgctcaggcgtgggggtagccgtcttaaacggccttatttacgccgtcggaggttttgccaccttagagactgaatctggcgaattagtcccaaccgagctgaactccgtcgaagcgtatgatccagaacgcaatgagtggtctttggttgctcctctgtcgactcgtcgttcaggggtgggagtggcggtattataactcgagcgg

SEQ ID NO: 16 - protein, 322 aa, Artificial Sequence
  Synthetic Construct
MNGLIYAVGGYDGSPDGSTHLNSVEAYDPERNEWSLVAPLSTRRSGVGVAVLNGLIYAVGGFATLETESGELVPTELNSVEAYDPERNEWSLVAPLSTRRSGVGVAVLNGLIYAVGGYDGSPDGSTHLNSVEAYDPERNEWSLVAPLSTRRSGVGVAVLNGLIYAVGGFATLETESGELVPTELNSVEAYDPERNEWSLVAPLSTRRSGVGVAVLNGLIYAVGGYDGSPDGSTHLNSVEAYDPERNEWSLVAPLSTRRSGVGVAVLNGLIYAVGGFATLETESGELVPTELNSVEAYDPERNEWSLVAPLSTRRSGVGVAVL

SEQ ID NO: 17 - DNA, 872 bp, Artificial Sequence
  SAKE protein
  CDS (12)..(863)
gggaattccatatgggggggcttttatatgctgttggtggatatgatggaaacactcatcttaattctcttgaatgctataaccccgagaccaacgaatggagtccagtagctcctctttccgtgccacgttctggtattggtgttgctgttttggggggacttttgtatgcagtcgggggatacgacggcaatacccatctgaattcattagagtgttataaccctgagaccaatgaatggtctccagtagctcctctgtcagtgccacgttccggtatcggggtagcggtgctgggtggtctgctgtacgcggtgggaggatacgatggcaatacgcatttaaattctttggagtgctataaccccgaaacaaacgagtggtctcccgtcgcacccctgtcggtaccgagatcaggcataggcgtcgctgtgcttgggggactgttatacgctgtcggtggttatgatggaaatacgcaccttaacagccttgaatgttacaatccggaaacaaatgaatggtccccggtagctcccttgtcggtcccccgttcgggcataggggtagctgtgttaggaggattgttgtatgcagtgggtgggtatgacggtaatacacacctgaactcattagagtgctataaccccgagaccaacgagtggtcgccagttgctcccttgtcagttccccggtccggaatcggggtcgctgtcttgggagggcttttgtatgcggtcgggggctatgatggtaatactcacctgaattcgcttgaatgctataatccggaaactaacgaatggtctccggttgcacctctgtcggtaccgcgtagtggcattggcgtggcagtattataactcgagcgg

SEQ ID NO: 18 - protein, 283 aa, Artificial Sequence
  Synthetic Construct
MGGLLYAVGGYDGNTHLNSLECYNPETNEWSPVAPLSVPRSGIGVAVLGGLLYAVGGYDGNTHLNSLECYNPETNEWSPVAPLSVPRSGIGVAVLGGLLYAVGGYDGNTHLNSLECYNPETNEWSPVAPLSVPRSGIGVAVLGGLLYAVGGYDGNTHLNSLECYNPETNEWSPVAPLSVPRSGIGVAVLGGLLYAVGGYDGNTHLNSLECYNPETNEWSPVAPLSVPRSGIGVAVLGGLLYAVGGYDGNTHLNSLECYNPETNEWSPVAPLSVPRSGIGVAVL

SEQ ID NO: 19 - DNA, 872 bp, Artificial Sequence
  SAKE protein
  CDS (12)..(863)
gggaattccatatgaatggacacatatatgcagttggtggctatgacggacatacccatttaaactcagttgaggcttatgacccggagaccgatgaatggcgcttggtcgcaccgttgacgacgcccagatccggtatgggagttgctgttcttaacggccatatatatgcggtaggcgggtatgatggtcatacccacctgaattccgtagaggcctatgatccagagactgacgagtggagacttgttgcccctttaacgacaccacggtcgggcatgggggtcgccgtccttaacggtcacatatacgcagtcggcggctatgatggtcatacccacctgaatagtgtggaagcttacgatccagaaacggacgaatggcgcttagttgctccgttgacgacacccagaagcgggatgggtgtggctgtgctgaacggccatatatatgcagtaggtgggtacgatggacacacacatcttaattccgtggaagcctatgatcccgaaactgatgagtggcggcttgtagctccactgacgaccccacgcagcgggatgggggtagctgttctgaacggccatatttacgcggtggggggctatgacggccatacgcatttaaattctgtcgaggcatacgacccagagacagatgaatggcgcctggtagcacctcttactacacctagatctggcatgggagtcgcggttttgaatgggcacatctacgccgtggggggctacgatggacatacacatttgaattctgtcgaagcttatgatcccgagacagatgaatggagactggttgccccattgaccacgccccggagtggaatgggcgtagctgtactttaactcgagcgg

SEQ ID NO: 20 - protein, 283 aa, Artificial Sequence
  Synthetic Construct
MNGHIYAVGGYDGHTHLNSVEAYDPETDEWRLVAPLTTPRSGMGVAVLNGHIYAVGGYDGHTHLNSVEAYDPETDEWRLVAPLTTPRSGMGVAVLNGHIYAVGGYDGHTHLNSVEAYDPETDEWRLVAPLTTPRSGMGVAVLNGHIYAVGGYDGHTHLNSVEAYDPETDEWRLVAPLTTPRSGMGVAVLNGHIYAVGGYDGHTHLNSVEAYDPETDEWRLVAPLTTPRSGMGVAVLNGHIYAVGGYDGHTHLNSVEAYDPETDEWRLVAPLTTPRSGMGVAVL

SEQ ID NO: 21 - protein, 285 aa, Homo sapiens
GRLIYTAGGYFRQSLSYLEAYNPSNGTWLRLADLQVPRSGLAGCVVGGLLYAVGGRNNSPDGNTDSSALDCYNPMTNQWSPCAPMSVPRNRIGVGVIDGHIYAVGGSHGCIHHNSVERYEPERDEWHLVAPMLTRRIGVGVAVLNRLLYAVGGFDGTNRLNSAECYYPERNEWRMITAMNTIRSGAGVCVLHNCIYAAGGYDGQDQLNSVERYDVETETWTFVAPMKHRRSALGITVHQGRIYVLGGYDGHTFLDSVECYDPDTDTWSEVTRMTSGRSGVGVAVT

SEQ ID NO: 22 - protein, 51 aa, Artificial Sequence
  S6AE (S6_2E) blade
DGRIYAVGGYDGSPDGHTHLNSVEAYDPETDTWSLVAPMKTRRSGVGVAVL

SEQ ID NO: 23 - protein, 51 aa, Artificial Sequence
  S6AR (S6_2R) blade
NRLLYAVGGYDGSPDGHTHLNSVECYDPETNEWSLVAPMNTRRSGVGVAVL

SEQ ID NO: 24 - protein, 51 aa, Artificial Sequence
  S6AC (S6_2C) blade
NGRIYAVGGYDGSPDGHTHLNSVEAYDPETDEWSFVAPMTTPRSGVGVAVL

SEQ ID NO: 25 - protein, 47 aa, Artificial Sequence
  S6BE (S6_6E) blade
NGLIYAVGGYDGNTHLNSVEAYDPERNEWSLVAPLSTRRSGVGVAVL

SEQ ID NO: 26 - protein, 94 aa, Artificial Sequence
  S6BE-3HH (S6_6E-3HH) blade 1 & blade 2
NGLIYAVGGYDGNTHLNSVEAYDPERNEWSLVAPLSTRRSGVGVAVLNGLIYAVGGYDGNTHLNSVEAYDPHHNEWSLVAPLSTRRSGVGVAVL

SEQ ID NO: 27 - protein, 50 aa, Artificial Sequence
  S6BE-L1 (S6_6E-L1) blade
NGLIYAVGGYDGTGYNTHLNSVEAYDPERNEWSLVAPLSTRRSGVGVAVL

SEQ ID NO: 28 - protein, 53 aa, Artificial Sequence
  S6BE-L2 (S6_6E-L2) blade
NGLIYAVGGYDGSPDYSTGTHLNSVEAYDPERNEWSLVAPLSTRRSGVGVAVL

SEQ ID NO: 29 - protein, 107 aa, Artificial Sequence
  S6BE-L3 (S6_6E-L3)  blade 1 & blade 2
NGLIYAVGGYDGSPDGSTHLNSVEAYDPERNEWSLVAPLSTRRSGVGVAVLNGLIYAVGGFATLETESGELVPTELNSVEAYDPERNEWSLVAPLSTRRSGVGVAVL

SEQ ID NO: 30 - protein, 47 aa, Artificial Sequence
  S6BR (S6_6R)
GGLLYAVGGYDGNTHLNSLECYNPETNEWSPVAPLSVPRSGIGVAVL

SEQ ID NO: 31 - protein, 47 aa, Artificial Sequence
  S6BC (does not express) (S6_6C)
NGHIYAVGGYDGHTHLNSVEAYDPETDEWRLVAPLTTPRSGMGVAVL

SEQ ID NO: 32 - protein, 42 aa, Artificial Sequence
  blade of variable length
  MISC_FEATURE (1)..(10): X at  position 10 can be 1 to 15 of any natural amino acids
NGRIYAVGGXLNSVEAYDPETDEWSFVAPMTTPRSGVGVAVL

SEQ ID NO: 33 - protein, 47 aa, Artificial Sequence; identical to SEQ ID NO: 25
  consensus sequence